European Patent Specification EP 3 455 371 B1, published January 18, 2023. Title: TISSUE-SPECIFIC EXOSOMES AS BIOMARKERS. Applicant: Helmholtz Zentrum Muenchen. The sequence listing filed with the application follows.

SEQUENCE LISTING (66 sequences)

SEQ ID NO: 1 - protein, 7 aa, Artificial sequence
  CDR1 in the VH domain of antibody 23A11
GFTFTDF

SEQ ID NO: 2 - protein, 8 aa, Artificial sequence
  CDR2 in the VH domain of antibody 23A11
RNKANGYT

SEQ ID NO: 3 - protein, 13 aa, Artificial sequence
  CDR3 in the VH domain of antibody 23A11
GGFDVYSGLLPDY

SEQ ID NO: 4 - protein, 17 aa, Artificial sequence
  CDR1 in the VL domain of antibody 23A11
KSSQNLLYRGNQKNYLA

SEQ ID NO: 5 - protein, 7 aa, Artificial sequence
  CDR2 in the VL domain of antibody 23A11
WTSTRQP

SEQ ID NO: 6 - protein, 9 aa, Artificial sequence
  CDR3 in the VL domain of antibody 23A11
QQYYGTPFT

SEQ ID NO: 7 - protein, 7 aa, Artificial sequence
  CDR1 in the VH domain of antibody 15G1
GFNFNDY

SEQ ID NO: 8 - protein, 8 aa, Artificial sequence
  CDR2 in the VH domain of antibody 15G1
RNKHYNYA

SEQ ID NO: 9 - protein, 9 aa, Artificial sequence
  CDR3 in the VH domain of antibody 15G1
SSYLRYFDF

SEQ ID NO: 10 - protein, 11 aa, Artificial sequence
  CDR1 in the VL domain of antibody 15G1
QASQDIGNWLA

SEQ ID NO: 11 - protein, 7 aa, Artificial sequence
  CDR2 in the VL domain of antibody 15G1
DATTLAD

SEQ ID NO: 12 - protein, 9 aa, Artificial sequence
  CDR3 in the VL domain of antibody 15G1
QQASSAPWT

SEQ ID NO: 13 - protein, 7 aa, Artificial sequence
  CDR1 in the VH domain of antibody 14H5
GFTFTGY

SEQ ID NO: 14 - protein, 6 aa, Artificial sequence
  CDR2 in the VH domain of antibody 14H5
NTGSGG

SEQ ID NO: 15 - protein, 9 aa, Artificial sequence
  CDR3 in the VH domain of antibody 14H5
TYWRRYFDY

SEQ ID NO: 16 - protein, 11 aa, Artificial sequence
  CDR1 in the VL domain of antibody 14H5
QASQDIGNWLA

SEQ ID NO: 17 - protein, 7 aa, Artificial sequence
  CDR2 in the VL domain of antibody 14H5
GATSLAD

SEQ ID NO: 18 - protein, 9 aa, Artificial sequence
  CDR3 in the VL domain of antibody 14H5
QQASSAPLT

SEQ ID NO: 19 - protein, 143 aa, Artificial sequence
  Variable domain heavy chain 23A11
MKLWLNWIFLLTLLNGIQCEVKLLESGGGLVQPGGSMRLSCAASGFTFTDFYMNWIRQPSGKAPEWLGFIRNKANGYTTESNPSVKGRFTISRDNTQSMLYLQMNTLRVEDTATYYCARGGFDVYSGLLPDYWGQGVMVTVSS

SEQ ID NO: 20 - protein, 133 aa, Artificial sequence
  Variable domain light chain 23A11
MESQTQVLMSLLLWISGTCGDIVMTQSPSSLAVSAGETVTINCKSSQNLLYRGNQKNYLAWYQQKPGQSPKLLIFWTSTRQPGVPDRFIGSGSGTDFTLTISSVQAEDLAIYYCQQYYGTPFTFGSGTKLEIR

SEQ ID NO: 21 - protein, 139 aa, Artificial sequence
  Variable domain heavy chain 15G1
MKLWLSWIFLVVLFKGVRCEVQILETGGGLVKPGGSLRLSCATSGFNFNDYFMNWVRQAPGKGLEWVAQIRNKHYNYATYYGESLEGRVTISRDDSKSNVYLQVNSLRPEDTAIYYCSRSSYLRYFDFWGPGTMVTVSS

SEQ ID NO: 22 - protein, 128 aa, Artificial sequence
  Variable domain light chain 15G1
MNVPTQLLGLLILWLTGGKCDIQMTQSPASLSASLEEIVTITCQASQDIGNWLAWYQQKPGKSPQLLIYDATTLADGVPSRFSGSRSGTQFSLKISRLQVEDIGIYYCQQASSAPWTFGGGTNLELKR

SEQ ID NO: 23 - protein, 137 aa, Artificial Sequence
  Variable domain heavy chain 14H5
MEWNWVFLFLLSVTAEVHSQVQLQQSGAELAKPGSSVKISCKASGFTFTGYYISWIKQTTGQGLDYIGYINTGSGGTNYNEKFKGKATLTVDKSSSTAFMQLSSLTPDDSAVYYCARTYWRRYFDYWGQGVMVTVSS

SEQ ID NO: 24 - protein, 128 aa, Artificial sequence
  Variable domain light chain 14H5
MNVPTQLLGLLILWLTGGKCDIQMTQSPASLSVSLEKIVTITCQASQDIGNWLAWYQQKPGKSPQLLIYGATSLADGVPSRFSGSRSGTQYSLKISRLQVEDIGIYYCQQASSAPLTFGSGTKLEIKR

SEQ ID NO: 25 - protein, 25 aa, Artificial sequence
  Framework region 1 variable domain heavy chain 23A11
EVKLLESGGGLVQPGGSMRLSCAAS

SEQ ID NO: 26 - protein, 19 aa, Artificial sequence
  Framework region 2 variable domain heavy chain 23A11
YMNWIRQPSGKAPEWLGFI

SEQ ID NO: 27 - protein, 41 aa, Artificial Sequence
  Framework region 3 variable domain heavy chain 23A11
TESNPSVKGRFTISRDNTQSMLYLQMNTLRVEDTATYYCAR

SEQ ID NO: 28 - protein, 11 aa, Artificial sequence
  Framework region 4 variable domain heavy chain 23A11
WGQGVMVTVSS

SEQ ID NO: 29 - protein, 23 aa, Artificial sequence
  Framework region 1 variable domain light chain 23A11
DIVMTQSPSSLAVSAGETVTINC

SEQ ID NO: 30 - protein, 15 aa, Artificial sequence
  Framework region 2 variable domain light chain 23A11
WYQQKPGQSPKLLIF

SEQ ID NO: 31 - protein, 32 aa, Artificial sequence
  Framework region 3 variable domain light chain 23A11
GVPDRFIGSGSGTDFTLTISSVQAEDLAIYYC

SEQ ID NO: 32 - protein, 10 aa, Artificial sequence
  Framework region 4 variable domain light chain 23A11
FGSGTKLEIR

SEQ ID NO: 33 - protein, 25 aa, Artificial sequence
  Framework region 1 variable domain heavy chain 15G1
EVQILETGGGLVKPGGSLRLSCATS

SEQ ID NO: 34 - protein, 19 aa, Artificial sequence
  Framework region 2 variable domain heavy chain 15G1
FMNWVRQAPGKGLEWVAQI

SEQ ID NO: 35 - protein, 41 aa, Artificial sequence
  Framework region 3 variable domain heavy chain 15G1
TYYGESLEGRVTISRDDSKSNVYLQVNSLRPEDTAIYYCSR

SEQ ID NO: 36 - protein, 11 aa, Artificial sequence
  Framework region 4 variable domain heavy chain 15G1
WGPGTMVTVSS

SEQ ID NO: 37 - protein, 23 aa, Artificial sequence
  Framework region 1 variable domain light chain 15G1
DIQMTQSPASLSASLEEIVTITC

SEQ ID NO: 38 - protein, 15 aa, Artificial sequence
  Framework region 2 variable domain light chain 15G1
WYQQKPGKSPQLLIY

SEQ ID NO: 39 - protein, 32 aa, Artificial sequence
  Framework region 3 variable domain light chain 15G1
GVPSRFSGSRSGTQFSLKISRLQVEDIGIYYC

SEQ ID NO: 40 - protein, 10 aa, Artificial sequence
  Framework region 4 variable domain light chain 15G1
FGGGTNLELK

SEQ ID NO: 41 - protein, 25 aa, Artificial sequence
  Framework region 1 variable domain heavy chain 14H5
QVQLQQSGAELAKPGSSVKISCKAS

SEQ ID NO: 42 - protein, 19 aa, Artificial sequence
  Framework region 2 variable domain heavy chain 14H5
YISWIKQTTGQGLDYIGYI

SEQ ID NO: 43 - protein, 41 aa, Artificial sequence
  Framework region 3 variable domain heavy chain 14H5
TNYNEKFKGKATLTVDKSSSTAFMQLSSLTPDDSAVYYCAR

SEQ ID NO: 44 - protein, 11 aa, Artificial sequence
  Framework region 4 variable domain heavy chain 14H5
WGQGVMVTVSS

SEQ ID NO: 45 - protein, 23 aa, Artificial sequence
  Framework region 1 variable domain light chain 14H5
DIQMTQSPASLSVSLEKIVTITC

SEQ ID NO: 46 - protein, 15 aa, Artificial sequence
  Framework region 2 variable domain light chain 14H5
WYQQKPGKSPQLLIY

SEQ ID NO: 47 - protein, 32 aa, Artificial sequence
  Framework region 3 variable domain light chain 14H5
GVPSRFSGSRSGTQYSLKISRLQVEDIGIYYC

SEQ ID NO: 48 - protein, 12 aa, Artificial sequence
  Framework region 4 variable domain light chain 14H5
FGSGTKLEIKRA

SEQ ID NO: 49 - DNA, 22 bp, artificial
  Primer
agattcgggatatgctgttggc

SEQ ID NO: 50 - DNA, 21 bp, artificial
  Primer
tcgggtcctagaccagtgttc

SEQ ID NO: 51 - DNA, 22 bp, artificial
  Primer
ctccaagccaaagtccttagag

SEQ ID NO: 52 - DNA, 22 bp, artificial
  Primer
aggagctgtcattagggacatc

SEQ ID NO: 53 - DNA, 21 bp, artificial
  Primer
agagaccaggtgaagtcagag

SEQ ID NO: 54 - DNA, 23 bp, artificial
  Primer
agtctgtgtagttagaagctcca

SEQ ID NO: 55 - DNA, 20 bp, artificial
  Primer
ctctggagagcacagtggag

SEQ ID NO: 56 - DNA, 19 bp, artificial
  Primer
acttccgagccgttgttct

SEQ ID NO: 57 - DNA, 19 bp, artificial
  Primer
atggtcaaccccaccgtgt

SEQ ID NO: 58 - DNA, 25 bp, artificial
  Primer
tttctgctgtctttggaactttgtc

SEQ ID NO: 59 - DNA, 21 bp, artificial
  Primer
ccctccactgtaacgaagact

SEQ ID NO: 60 - DNA, 20 bp, artificial
  Primer
cagtggtccagtcaacgagt

SEQ ID NO: 61 - DNA, 20 bp, artificial
  Primer
ccccgctactactccatcag

SEQ ID NO: 62 - DNA, 20 bp, artificial
  Primer
ccactgacacttcgcacaaa

SEQ ID NO: 63 - DNA, 22 bp, artificial
  Primer
agccgtgaccactgacaacgag

SEQ ID NO: 64 - DNA, 23 bp, artificial
  Primer
gctgcatggttctgagtgctaag

SEQ ID NO: 65 - DNA, 20 bp, artificial
  Primer
ggcctctacgactcagtcca

SEQ ID NO: 66 - DNA, 20 bp, artificial
  Primer
taagccggctgagatcttgt